European Patent Application EP 4 151 657 A1, published March 22, 2023. Title: RECOMBINANT HUMAN ANTIBODIES THAT INHIBIT THE HUMAN TISSUE KALLIKREIN 7 (KLK7) AND THEIR USE AGAINST DISEASES THAT CAUSE DESQUAMATION OF THE SKIN. Applicant: Fundacao Universidade Federal do ABC - UFABC. The sequence listing filed with the application follows.

SEQUENCE LISTING (26 sequences)

SEQ ID NO: 1 - DNA, 804 bp, Artificial sequence
  antibody
ccatggcccaggtacagctgcagcagtcaggcccaggactggtgcagccttcggagaccctgtccctcacgtgcactgtctctggtggctccatgaatagttactattggagctggatccggcagcccgccgggaagggactggagtggatcgggcgtgtctatcccactgggggaaccgactacaacccctccctcaagagtcgagtcataatgtcagtagacacggttcggaaccacttctccctgagattgaactctgtgaccgccgcggactcggccgtgtattactgtgcgagagatcggggctacagtaactacggctggttcgacccctggggccagggaaccctggtcaacgtctcctcagggagtgcatccgccccaaagcttgaagaaggtgaattttcagaagcacgcgtaaattttatgctgactcagccccactctgtgtcggcgtctccggggaagacggtaaccatctcctgcaccggcagcagtggcagcattgccagcaactttgtacagtggtaccagcagcgcccgggcagtgcccccaccactgtgatctatgaagataatcaaagaccctctggggtccctgatcggttctccggctccatcgacagttcgtccaactctgcctccctcagcatctctggactgcagactgacgacgaggctgactactactgtcagtcttctgatagcagcaatcacgtggtgttcggcggagggaccaagctgaccgtcctaggtcagcccaaggctgccccctcggtcactctgttcccaccgtcctctg

SEQ ID NO: 2 - protein, 498 aa, Artificial sequence
  antibody
MAQVQLQQSGPGLVQPSETLSLTCTVSGGSMNSYYWSWIRQPAGKGLEWIGRVYPTGGTDYNPSLKSRVIMSVDTVRNHFSLRLNSVTAADSAVYYCARDRGYSNYGWFDPWGQGTLVNVSSGSASAPKLEEGEFSEARVNFMLTQPHSVSASPGKTVTISCTGSSGSIASNFVQWYQQRPGSAPTTVIYEDNQRPSGVPDRFSGSIDSSSNSASLSISGLQTDDEADYYCQSSDSSNHVVFGGGTKLTVLGQPKAAPSVTLFPPSSAAASDKTHTCPPCPAPELLGGPSVFLFPPKPKDTLMISRTPEVTCVVVDVSHEDPEVKFNWYVDGVEVHNAKTKPREEQYNSTYRVVSVLTVLHQDWLNGKEYKCKVSNKALPAPIEKTISKAKGQPREPQVYTLPPSREEVTKNQVSLTCLVKGFYPSDIAVEWESNGQPENNYKTTPPVLDSDGSFFLYSKLTVDKSRWQQGNVFSCSVMHEALHNHYTQKSLSLSPGK

SEQ ID NO: 3 - DNA, 801 bp, Artificial sequence
  antibody
ccatggcccaggttcagctggtgcagtctgggggaggcgtggtccagcctgggaggtccctgagactctcctgtgcagcctctggattcatcttcagtgattattctatgcattgggtccgccaggctccaggcaaggggctggagtgggtggcagttatgtcatatgatgcaaggagtcaattctacgcagactccgtgaagggccgattcaccatctccagagacaattccaagaacactctatatctgcaaatgaacagcctgagagaggaagacacggctgtgtattactgtgcgacagatgttggcaattccccgtttgactactggggccagggaaccctggtcaccgtctcctcagggagtgcatccgccccaaagcttgaagaaggtgaattttcagaagcacgcgtacaggctgtgctgactcagcccccctcagtgtctggggccctagggcagagggtcaccatctcctgcactgggagcagctccaacatcggggcgccttatgatgtacactggtaccagcagcttccaggaacagcccccaaactcctcatatacggtaataacaatcggccctcaggggtccctgaccgattctctggctccaagtctggcacctcagcctccctggccatcagtgggctccggtccgaggatgaggctgattattactgtgcagcatgggatgacagcctgagtggttcttgggtgttcggcggagggaccaagctgaccgtcctaggtcagcccaaggctgccccctcggtcactctgttcccaccgtcctctg

SEQ ID NO: 4 - protein, 497 aa, Artificial sequence
  antibody
MAQVQLVQSGGGVVQPGRSLRLSCAASGFIFSDYSMHWVRQAPGKGLEWVAVMSYDARSQFYADSVKGRFTISRDNSKNTLYLQMNSLREEDTAVYYCATDVGNSPFDYWGQGTLVTVSSGSASAPKLEEGEFSEARVQAVLTQPPSVSGALGQRVTISCTGSSSNIGAPYDVHWYQQLPGTAPKLLIYGNNNRPSGVPDRFSGSKSGTSASLAISGLRSEDEADYYCAAWDDSLSGSWVFGGGTKLTVLGQPKAAPSVTLFPPSSAAASDKTHTCPPCPAPELLGGPSVFLFPPKPKDTLMISRTPEVTCVVVDVSHEDPEVKFNWYVDGVEVHNAKTKPREEQYNSTYRVVSVLTVLHQDWLNGKEYKCKVSNKALPAPIEKTISKAKGQPREPQVYTLPPSREEVTKNQVSLTCLVKGFYPSDIAVEWESNGQPENNYKTTPPVLDSDGSFFLYSKLTVDKSRWQQGNVFSCSVMHEALHNHYTQKSLSLSPGK

SEQ ID NO: 5 - DNA, 819 bp, Artificial sequence
  antibody
ccatggcccaggtgcagctgcaggagtccgggggaggcttggtaaagcctggggggtcccttagactctcctgtgcagcctctggattcactttcagtaacgcctggatgagctgggtccgccaggctccagggaaggggctggagtgggttggccgtattaaaagcaaaactgatggtgggacaacagactacgctgcacccgtgaaaggcagattcaccatctcaagagatgattcaaaaaacacgctgtatctgcaaatgaacagcctgaaaaccgaggacacagccgtgtattactgtaccacagggttggtcctttattgtggtggtgactgctatccgtttgactactggggccagggaaccctggtcaccgtctcctcagggagtgcatccgccccaaagcttgaagaaggtgaattttcagaagcacgcgtactgcctgtgctgactcagccaccctcagcgtctgggacccccgggcagagggtcaccatctcttgttctggaagcagctccaacatcgaaacaaatactttgagctggtaccaacaactcccaggaagggcccccaaactcctcatgcataatgataatgagcggcccccaggggtccctgaccgattctctggctccaagtctggcacctcagcctccctggccatcagtgggctccaatctgaggatgaggctgattattactgtgcagcatgggatgacagtttgaatggtcaggtgttcggcggagggaccaaggtgaccgtcttaggtcagcccaaggctgccccctcggtcactctgttcccgccgtcctctg

SEQ ID NO: 6 - protein, 503 aa, Artificial sequence
  antibody
MAQVQLQESGGGLVKPGGSLRLSCAASGFTFSNAWMSWVRQAPGKGLEWVGRIKSKTDGGTTDYAAPVKGRFTISRDDSKNTLYLQMNSLKTEDTAVYYCTTGLVLYCGGDCYPFDYWGQGTLVTVSSGSASAPKLEEGEFSEARVLPVLTQPPSASGTPGQRVTISCSGSSSNIETNTLSWYQQLPGRAPKLLMHNDNERPPGVPDRFSGSKSGTSASLAISGLQSEDEADYYCAAWDDSLNGQVFGGGTKVTVLGQPKAAPSVTLFPPSSAAASDKTHTCPPCPAPELLGGPSVFLFPPKPKDTLMISRTPEVTCVVVDVSHEDPEVKFNWYVDGVEVHNAKTKPREEQYNSTYRVVSVLTVLHQDWLNGKEYKCKVSNKALPAPIEKTISKAKGQPREPQVYTLPPSREEVTKNQVSLTCLVKGFYPSDIAVEWESNGQPENNYKTTPPVLDSDGSFFLYSKLTVDKSRWQQGNVFSCSVMHEALHNHYTQKSLSLSPGK

SEQ ID NO: 7 - DNA, 795 bp, Artificial sequence
  antibody
ccatggcccaggtccagctggtgcagtctggggctgaggtgaagaagcctggggctacagtgaaaatctcctgcaaggtttctggatacaccttcaccgactactacatgcactgggtgcaacaggcccctggaaaagggcttgagtggatgggacttgttgatcctgaagatggtgaaacaatatacgcagagaagttccagggcagagtcaccataaccgcggacacgtctacagacacagcctacatggagctgagcagcctgagatctgaggacacggccgtgtattactgtgcaacaggcaatgtacgtaggatagactactggggccagggaaccctggtcaccgtctcctcagggagtgcatccgccccaaagcttgaagaaggtgaattttcagaagcacgcgtaaattttatgctgactcagccccactctgtgtcggagtctccggggaagacggtaaccatctcctgcaccggcagcagtggcagcattgccgacaactatgtgcagtggtaccagcagcgcccgggcagtgcccccatcaatgtgatctatgaggataaccaaagaccctctggggtccctgatcggttctctggctccatcgacagctcctccaactctgcctccctcaccatctctggactgaagactgaggacgaggctgactactactgtcagtcttatgatagcagcaatcatgtggtattcggcggagggaccaagctgaccgtcctaggtcagcccaaggctgccccctcggtcactctgttcccaccgtcttctg

SEQ ID NO: 8 - protein, 495 aa, Artificial sequence
  antibody
MAQVQLVQSGAEVKKPGATVKISCKVSGYTFTDYYMHWVQQAPGKGLEWMGLVDPEDGETIYAEKFQGRVTITADTSTDTAYMELSSLRSEDTAVYYCATGNVRRIDYWGQGTLVTVSSGSASAPKLEEGEFSEARVNFMLTQPHSVSESPGKTVTISCTGSSGSIADNYVQWYQQRPGSAPINVIYEDNQRPSGVPDRFSGSIDSSSNSASLTISGLKTEDEADYYCQSYDSSNHVVFGGGTKLTVLGQPKAAPSVTLFPPSSAAASDKTHTCPPCPAPELLGGPSVFLFPPKPKDTLMISRTPEVTCVVVDVSHEDPEVKFNWYVDGVEVHNAKTKPREEQYNSTYRVVSVLTVLHQDWLNGKEYKCKVSNKALPAPIEKTISKAKGQPREPQVYTLPPSREEVTKNQVSLTCLVKGFYPSDIAVEWESNGQPENNYKTTPPVLDSDGSFFLYSKLTVDKSRWQQGNVFSCSVMHEALHNHYTQKSLSLSPGK

SEQ ID NO: 9 - DNA, 783 bp, Artificial sequence
  antibody
ccatggcccaagtccagctggtgcagtctggggctgaggtgaagaggcctggggcctcagtgaaggtctcctgcaaggtttccggatacaccctcactgaattatccatgcactgggtgcgacaggctcctggaaaagggcttgagtggatgggaggttttgatcctgaagatggtgaaacaatctacgcacagaagttccagggcagagtcaccatgaccgaggacacatctacagacacagcctacatggagctgagcagcctgagatctgaggacacggccgtgtattactgtgcaacattgaggcagtggctagaatttgactactggggccagggaaccctggtcaccgtctcctcagggagtgcatccgccccaaagcttgaagaaggtgaattttcagaagcacgcgtacagtctgtgttgacgcagccgccctcagtgtccgtgtccccaggacagacagccagcatcacctgctctggagatagattgggggataaatatgcttcctggtatcagcagaagccaggccagtcccctgtgctggtcatctatcaagataccaagcggccctcagggatccctgagcgattctctggctccaactctgggaacacagccactctgaccatcagcgggacccaggctatggatgaggctgactattactgtcaggcgtgggacagcagcactgcggtattcggcggcgggaccaagctgaccgtcctaggtcagcccaaggctgccccctcggtcactctgttcccaccgtcctctg

SEQ ID NO: 10 - protein, 491 aa, Artificial sequence
  antibody
MAQVQLVQSGAEVKRPGASVKVSCKVSGYTLTELSMHWVRQAPGKGLEWMGGFDPEDGETIYAQKFQGRVTMTEDTSTDTAYMELSSLRSEDTAVYYCATLRQWLEFDYWGQGTLVTVSSGSASAPKLEEGEFSEARVQSVLTQPPSVSVSPGQTASITCSGDRLGDKYASWYQQKPGQSPVLVIYQDTKRPSGIPERFSGSNSGNTATLTISGTQAMDEADYYCQAWDSSTAVFGGGTKLTVLGQPKAAPSVTLFPPSSAAASDKTHTCPPCPAPELLGGPSVFLFPPKPKDTLMISRTPEVTCVVVDVSHEDPEVKFNWYVDGVEVHNAKTKPREEQYNSTYRVVSVLTVLHQDWLNGKEYKCKVSNKALPAPIEKTISKAKGQPREPQVYTLPPSREEVTKNQVSLTCLVKGFYPSDIAVEWESNGQPENNYKTTPPVLDSDGSFFLYSKLTVDKSRWQQGNVFSCSVMHEALHNHYTQKSLSLSPGK

SEQ ID NO: 11 - DNA, 792 bp, Artificial sequence
  antibody
ccatggcccagctgcagctacagcagtccggcccaggactggtgaagccttcggggaccctgtccctcacctgcgctgtctctggtggctccatcagcagtagtaactggtggagttgggtccgccagcccccagggaaggggctggagtggattggggaaatctatcatagtgggagcaccaactacaacccgtccctcaagagtcgagtcaccatatcagtagacaagtccaagaaccagttctccctgaagctgagctctgtgaccgccgcggacacggccgtgtattactgtgcgacaggtacggccagcttaatcggtatggacgtctggggccaagggaccacggtcaccgtctcctcagggagtgcatccgccccaaagcttgaagaaggtgaattttcagaagcacgcgtatcctatgtgctgactcagccaccctcggtgtcagtggccccaggacagacggccaggattccctgtgggggaaataacattggagataaaaatgtgcagtggtaccagcagaagccagaccaggcccctgtgctggtcgtctatgatgatagcgaccggccctcaggcatccctgagcgattctctggctccaactctgggaacaaggccgccctgaccatcagcggggtcgaggtcggggatgaggccgactattattgtcaggtgtgggataggagttctgatgtcgtggtcttcggcggagggaccaagctgaccgtcctaggtcagcccaaggctgccccctcggtcactctgttcccaccctcctctg

SEQ ID NO: 12 - protein, 494 aa, Artificial sequence
  antibody
MAQLQLQQSGPGLVKPSGTLSLTCAVSGGSISSSNWWSWVRQPPGKGLEWIGEIYHSGSTNYNPSLKSRVTISVDKSKNQFSLKLSSVTAADTAVYYCATGTASLIGMDVWGQGTTVTVSSGSASAPKLEEGEFSEARVSYVLTQPPSVSVAPGQTARIPCGGNNIGDKNVQWYQQKPDQAPVLVVYDDSDRPSGIPERFSGSNSGNKAALTISGVEVGDEADYYCQVWDRSSDVVVFGGGTKLTVLGQPKAAPSVTLFPPSSAAASDKTHTCPPCPAPELLGGPSVFLFPPKPKDTLMISRTPEVTCVVVDVSHEDPEVKFNWYVDGVEVHNAKTKPREEQYNSTYRVVSVLTVLHQDWLNGKEYKCKVSNKALPAPIEKTISKAKGQPREPQVYTLPPSREEVTKNQVSLTCLVKGFYPSDIAVEWESNGQPENNYKTTPPVLDSDGSFFLYSKLTVDKSRWQQGNVFSCSVMHEALHNHYTQKSLSLSPGK

SEQ ID NO: 13 - DNA, 798 bp, Artificial sequence
  antibody
ccatggccgaggtgcagctggtggagtctggggctgaggtgaagaagcctggggcctcagtgaaggtctcctgcaaggtttccggatacaccctcactgaattatccatgcactgggtgcgacagactcctggaaaagggcttgagtggatgggaggttttgatcctgaagatggtgaaacaatctacgcacagaagttccagggcagagtcaccatgaccgaggacacatctacagacacagcctacatggagctgagcagcctgagatctgaggacacggccgtgtattactgtgcaacccaaggatatagtggctacgattactactttgactactggggccagggaaccctggtcaccgtctcctcagggagtgcatccgccccaaagcttgaagaaggtgaattttcagaagcacgcgtatcttctgagctgactcaggaccctattgtgtctgtggccttgggacagacagtcaggatcgcttgccaaggagacagcctcagaacctcttatgcaagctggtaccagcagaagccaggacaggcccctgtacttgtcatgtacggtaaaaacaatcggccctcagggatccccgaccgattctctggctcctactcagggatctcagcttccttgaccatcactggggctcaggcggaagatgaggctgactattactgttactcccgggagaccactggataccattatgtcttcggaactgggaccaaggtcaccgtcctaggtcagcccaaggccaaccccactgtcactctgttcccaccctcctctg

SEQ ID NO: 14 - protein, 496 aa, Artificial sequence
  antibody
MAEVQLVESGAEVKKPGASVKVSCKVSGYTLTELSMHWVRQTPGKGLEWMGGFDPEDGETIYAQKFQGRVTMTEDTSTDTAYMELSSLRSEDTAVYYCATQGYSGYDYYFDYWGQGTLVTVSSGSASAPKLEEGEFSEARVSSELTQDPIVSVALGQTVRIACQGDSLRTSYASWYQQKPGQAPVLVMYGKNNRPSGIPDRFSGSYSGISASLTITGAQAEDEADYYCYSRETTGYHYVFGTGTKVTVLGQPKANPTVTLFPPSSAAASDKTHTCPPCPAPELLGGPSVFLFPPKPKDTLMISRTPEVTCVVVDVSHEDPEVKFNWYVDGVEVHNAKTKPREEQYNSTYRVVSVLTVLHQDWLNGKEYKCKVSNKALPAPIEKTISKAKGQPREPQVYTLPPSREEVTKNQVSLTCLVKGFYPSDIAVEWESNGQPENNYKTTPPVLDSDGSFFLYSKLTVDKSRWQQGNVFSCSVMHEALHNHYTQKSLSLSPGK

SEQ ID NO: 15 - DNA, 805 bp, Artificial sequence
  antibody
ccatggcccaagtccagctggtacagtctggagcagaggtgaaaaagcccggggagtctctgaggatctcctgtaagggttctgaatacagctttaccacctcctggatcaactgggtgcgccagatgcccgggaaaggcctggagtggatggggaccattgatcctagtgactcttataccgactacagcccgtccttccgaggccacgtcaccatctcagttgacaagtccatcagtactgcctacctgcagtggagcagcctgaaggcctcagacaccgccgtctattactgtgcgactccgtatagcacttctcccgggtccggtttcgactcctggggccagggaaccctggtcaccgtctcctcagggagtgcatccgccccaaagcttgaagaaggtgaattttcagaagcacgcgtaaattttatgctgactcagccccactctgtgtcggggtctccggggaagacggttaccatctcctgtaccgccaacggtggcagccttgccaacaactttgtgcagtggtaccagcagcgcccgggcagtgcccccacccctgttatctatgaggatagtcaaagaccctctggggtccctgatcggttctctggcttcatcgacagctcctccaactctgcctccctcaccatctctggactgaagactgaggacgaggctgattactactgtcagtcttatgataacaaagattgggtgttcggcggagggaccaggctgaccgttcctgggtcagcccaaggctgccccctcggtcactctgttcccgccctcctctg

SEQ ID NO: 16 - protein, 498 aa, Artificial sequence
  antibody
MAQVQLVQSGAEVKKPGESLRISCKGSEYSFTTSWINWVRQMPGKGLEWMGTIDPSDSYTDYSPSFRGHVTISVDKSISTAYLQWSSLKASDTAVYYCATPYSTSPGSGFDSWGQGTLVTVSSGSASAPKLEEGEFSEARVNFMLTQPHSVSGSPGKTVTISCTANGGSLANNFVQWYQQRPGSAPTPVIYEDSQRPSGVPDRFSGFIDSSSNSASLTISGLKTEDEADYYCQSYDNKDWVFGGGTRLTVLGQPKAAPSVTLFPPSSAAASDKTHTCPPCPAPELLGGPSVFLFPPKPKDTLMISRTPEVTCVVVDVSHEDPEVKFNWYVDGVEVHNAKTKPREEQYNSTYRVVSVLTVLHQDWLNGKEYKCKVSNKALPAPIEKTISKAKGQPREPQVYTLPPSREEVTKNQVSLTCLVKGFYPSDIAVEWESNGQPENNYKTTPPVLDSDGSFFLYSKLTVDKSRWQQGNVFSCSVMHEALHNHYTQKSLSLSPGK

SEQ ID NO: 17 - DNA, 811 bp, Artificial sequence
  antibody
ccatggcccaggtccagctggtgcagtctggggctgaggtgaagaagcctggggcctcagtgaaggtctcctgcaaggtttccggatacaccctcactgaattatccatgcactgggtgcgccagactcctggaaaagggcttgagtggatgggaggttttgatcctgaagatggtgaaacaatctacgcacagaagttccagggcagagtcaccatgaccgaggacacatctacagacacagcctacatggagctgagcagcctgaggtctgaggacacggccgtgtattactgtgcaacccaaggatatagtggctacgattactactttgactactggggccagggaaccctggtcaccgtctcctcagggagtgcatccgccccaaagcttgaagaaggtgaattttcagaagcacgcgtacagtctgtgttgacgcagccgccctcagcgtctgggacccccgggcagagggtcaccatctcttgttctggaagcagctccaacatcggaagtaatgctgtaaactggtaccagcagctcccaggaacggcccccaaactcctcatctatagtaataatcaccggccctcaggggtccctgaccgattctctggctccaagtctggcacctcagcctccctggccatcagtggactccagtctgaggatgaggctgattattactgtgcagcatgggatgacggcctgaatggttgggtgttcggcggagggaccaagctgaccgtcctaggtcagcccaaggctgccccctcggtcactctgttcccaccgtcctctgcggccgc

SEQ ID NO: 18 - protein, 498 aa, Artificial sequence
  antibody
MAQVQLVQSGAEVKKPGASVKVSCKVSGYTLTELSMHWVRQTPGKGLEWMGGFDPEDGETIYAQKFQGRVTMTEDTSTDTAYMELSSLRSEDTAVYYCATQGYSGYDYYFDYWGQGTLVTVSSGSASAPKLEEGEFSEARVQSVLTQPPSASGTPGQRVTISCSGSSSNIGSNAVNWYQQLPGTAPKLLIYSNNHRPSGVPDRFSGSKSGTSASLAISGLQSEDEADYYCAAWDDGLNGWVFGGGTKLTVLGQPKAAPSVTLFPPSSAAASDKTHTCPPCPAPELLGGPSVFLFPPKPKDTLMISRTPEVTCVVVDVSHEDPEVKFNWYVDGVEVHNAKTKPREEQYNSTYRVVSVLTVLHQDWLNGKEYKCKVSNKALPAPIEKTISKAKGQPREPQVYTLPPSREEVTKNQVSLTCLVKGFYPSDIAVEWESNGQPENNYKTTPPVLDSDGSFFLYSKLTVDKSRWQQGNVFSCSVMHEALHNHYTQKSLSLSPGK

SEQ ID NO: 19 - DNA, 814 bp, Artificial sequence
  antibody
ccatggcccaggtccagctggtgcagtctggggctgaggtgaagaagcctggggcctcagtgaaggtctcctgcaaggtttccggatacaccctcactgaattatccatgcactgggtgcgccagactcctggaaaagggcttgagtggatgggaggttttgatcctgaagatggtgaaacaatctacgcacagaagttccagggcagagtcaccatgaccgaggacacatctacagacacagcctacatggagctgagcagcctgaggtctgaggacacggccgtgtattactgtgcaacccaaggatatagtggctacgattactactttgactactggggccagggaaccctggtcaccgtctcctcagggagtgcatccgccccaaagcttgaagaaggtgaattttcagaagcacgcgtacaggctgtggtgactcaggagccatcgttgtcagtgtcccctggagggacagtcacactcagttgtggattgagctctggctcagtctcttctactcattatcccagttggtaccagcagaccccaggccaggccccacgtacactcatctacaacacaaacattcgctcttctggggtccctgaccgattctctggctccaagtctggcacctcagcctccctggccatcagtgggctccggtccgaggatgaggctgattattactgtgcagcatgggatgacagcctgagtggttgggtgttcggcggagggaccaagctgaccgtcctaggtcagcccaaggctgccccctcggtcactctgttcccaccctcctctgcggccgc

SEQ ID NO: 20 - protein, 499 aa, Artificial sequence
  antibody
MAQVQLVQSGAEVKKPGASVKVSCKVSGYTLTELSMHWVRQTPGKGLEWMGGFDPEDGETIYAQKFQGRVTMTEDTSTDTAYMELSSLRSEDTAVYYCATQGYSGYDYYFDYWGQGTLVTVSSGSASAPKLEEGEFSEARVQAVVTQEPSLSVSPGGTVTLSCGLSSGSVSSTHYPSWYQQTPGQAPRTLIYNTNIRSSGVPDRFSGSKSGTSASLAISGLRSEDEADYYCAAWDDSLSGWVFGGGTKLTVLGQPKAAPSVTLFPPSSAAASDKTHTCPPCPAPELLGGPSVFLFPPKPKDTLMISRTPEVTCVVVDVSHEDPEVKFNWYVDGVEVHNAKTKPREEQYNSTYRVVSVLTVLHQDWLNGKEYKCKVSNKALPAPIEKTISKAKGQPREPQVYTLPPSREEVTKNQVSLTCLVKGFYPSDIAVEWESNGQPENNYKTTPPVLDSDGSFFLYSKLTVDKSRWQQGNVFSCSVMHEALHNHYTQKSLSLSPGK

SEQ ID NO: 21 - DNA, 811 bp, Artificial sequence
  antibody
ccatggcccaggtccagctggtgcagtctggggctgaggtgaagaagcctggggcctcagtgaaggtctcctgcaaggtttccggatacaccctcactgaattatccatgcactgggtgcgccagactcctggaaaagggcttgagtggatgggaggttttgatcctgaagatggtgaaacaatctacgcacagaagttccagggcagagtcaccatgaccgaggacacatctacagacacagcctacatggagctgagcagcctgaggtctgaggacacggccgtgtattactgtgcaacccaaggatatagtggctacgattactactttgactactggggccagggaaccctggtcaccgtctcctcagggagtgcatccgccccaaagcttgaagaaggtgaattttcagaagcacgcgtacaggctgtgctgactcagccaccctcagcgtctgggacccccgggcagagggtcaccatctcttgttctgggagcaactccaacgtcgggaggtatactgtaaactggtaccaacaactcccaggaacggcccccaaactcctcatcaatactaatgatcggcggccctcaggggtccctgaccgattctctggctccaagtctggcacctcagcctccctggccatcagtggcctccagtctgaggatgaggctgcttattactgtgcagcctgggatgacagccggaatggttgggcgttcggcggagggaccaagctgaccgtcctccgtcagcccaaggctgccccctcggtcactctgttcccgccctcctctgcggccgc

SEQ ID NO: 22 - protein, 498 aa, Artificial sequence
  antibody
MAQVQLVQSGAEVKKPGASVKVSCKVSGYTLTELSMHWVRQTPGKGLEWMGGFDPEDGETIYAQKFQGRVTMTEDTSTDTAYMELSSLRSEDTAVYYCATQGYSGYDYYFDYWGQGTLVTVSSGSASAPKLEEGEFSEARVQAVLTQPPSASGTPGQRVTISCSGSNSNVGRYTVNWYQQLPGTAPKLLINTNDRRPSGVPDRFSGSKSGTSASLAISGLQSEDEAAYYCAAWDDSRNGWAFGGGTKLTVLRQPKAAPSVTLFPPSSAAASDKTHTCPPCPAPELLGGPSVFLFPPKPKDTLMISRTPEVTCVVVDVSHEDPEVKFNWYVDGVEVHNAKTKPREEQYNSTYRVVSVLTVLHQDWLNGKEYKCKVSNKALPAPIEKTISKAKGQPREPQVYTLPPSREEVTKNQVSLTCLVKGFYPSDIAVEWESNGQPENNYKTTPPVLDSDGSFFLYSKLTVDKSRWQQGNVFSCSVMHEALHNHYTQKSLSLSPGK

SEQ ID NO: 23 - DNA, 805 bp, Artificial sequence
  antibody
ccatggcccaggtccagctggtgcagtctggggctgaggtgaagaagcctggggcctcagtgaaggtctcctgcaaggtttccggatacaccctcactgaattatccatgcactgggtgcgccagactcctggaaaagggcttgagtggatgggaggttttgatcctgaagatggtgaaacaatctacgcacagaagttccagggcagagtcaccatgaccgaggacacatctacagacacagcctacatggagctgagcagcctgaggtctgaggacacggccgtgtattactgtgcaacccaaggatatagtggctacgattactactttgactactggggccagggaaccctggtcaccgtctcctcagggagtgcatccgccccaaagcttgaagaaggtgaattttcagaagcacgcgtatcttctgagctgactcaggaccctgctgtgtctgtggccttgggacagacagtcaggatcacatgccaaggagacagcctcagaaactattatgcaagctggtaccagcagaagccaggacaggcccccgtagttgtcatctatggtaaaaacaaccggccctcagggatcccagaccgattctctggctccagctcaggaaacacagcttccttgaccatcactggggctcaagcggaagatgaggctgactattactgtaactcccgggacagcagtggtaaccatgtggtattcggcggagggaccaagctgaccgtcctaggtcagtccaaggctgccccctcggtcactctgttcccaccctcctctgcggccgc

SEQ ID NO: 24 - protein, 496 aa, Artificial sequence
  antibody
MAQVQLVQSGAEVKKPGASVKVSCKVSGYTLTELSMHWVRQTPGKGLEWMGGFDPEDGETIYAQKFQGRVTMTEDTSTDTAYMELSSLRSEDTAVYYCATQGYSGYDYYFDYWGQGTLVTVSSGSASAPKLEEGEFSEARVSSELTQDPAVSVALGQTVRITCQGDSLRNYYASWYQQKPGQAPVVVIYGKNNRPSGIPDRFSGSSSGNTASLTITGAQAEDEADYYCNSRDSSGNHVVFGGGTKLTVLGQSKAAPSVTLFPPSSAAASDKTHTCPPCPAPELLGGPSVFLFPPKPKDTLMISRTPEVTCVVVDVSHEDPEVKFNWYVDGVEVHNAKTKPREEQYNSTYRVVSVLTVLHQDWLNGKEYKCKVSNKALPAPIEKTISKAKGQPREPQVYTLPPSREEVTKNQVSLTCLVKGFYPSDIAVEWESNGQPENNYKTTPPVLDSDGSFFLYSKLTVDKSRWQQGNVFSCSVMHEALHNHYTQKSLSLSPGK

SEQ ID NO: 25 - DNA, 808 bp, Artificial sequence
  antibody
ccatggcccaggtccagctggtgcagtctggggctgaggtgaagaagcctggggcctcagtgaaggtctcctgcaaggtttccggatacaccctcactgaattatccatgcactgggtgcgccagactcctggaaaagggcttgagtggatgggaggttttgatcctgaagatggtgaaacaatctacgcacagaagttccagggcagagtcaccatgaccgaggacacatctacagacacagcctacatggagctgagcagcctgaggtctgaggacacggccgtgtattactgtgcaacccaaggatatagtggctacgattactactttgactactggggccagggaaccctggtcaccgtctcctcagggagtgcatccgccccaaagcttgaagaaggtgaattttcagaagcacgcgtatcttctgagctgactcaggaccctgctgtgtctgtggccttgggacagacagtcaggatcacatgccaaggagacagcctcagaagctattatgcaagctggtaccagcagaagccaggacaggcccctgtagttgtcatctatggtaaaaacgaccggccctcagggatcccagaccgattctctggctccagctcaggaaacacagcttccttgaccatcactggggctcaggcggaagatgaggctgactattactgtaactcccgggacagcagtggtaaccatcatgtggtattcggcggagggaccaagctgaccgtcctaggtcagcccaaggctgccccctcggtcactctgttcccaccgtcctctgcggccgc

SEQ ID NO: 26 - protein, 497 aa, Artificial sequence
  antibody
MAQVQLVQSGAEVKKPGASVKVSCKVSGYTLTELSMHWVRQTPGKGLEWMGGFDPEDGETIYAQKFQGRVTMTEDTSTDTAYMELSSLRSEDTAVYYCATQGYSGYDYYFDYWGQGTLVTVSSGSASAPKLEEGEFSEARVSSELTQDPAVSVALGQTVRITCQGDSLRSYYASWYQQKPGQAPVVVIYGKNDRPSGIPDRFSGSSSGNTASLTITGAQAEDEADYYCNSRDSSGNHHVVFGGGTKLTVLGQPKAAPSVTLFPPSSAAASDKTHTCPPCPAPELLGGPSVFLFPPKPKDTLMISRTPEVTCVVVDVSHEDPEVKFNWYVDGVEVHNAKTKPREEQYNSTYRVVSVLTVLHQDWLNGKEYKCKVSNKALPAPIEKTISKAKGQPREPQVYTLPPSREEVTKNQVSLTCLVKGFYPSDIAVEWESNGQPENNYKTTPPVLDSDGSFFLYSKLTVDKSRWQQGNVFSCSVMHEALHNHYTQKSLSLSPGK